European Patent Specification EP 4 121 092 B1, published April 24, 2024. Title: COMPOSITIONS AND METHODS RELATING TO THE TREATMENT OF DISEASES. Applicant: ILC Therapeutics LTD. The sequence listing filed with the application follows.

SEQUENCE LISTING (3 sequences)

SEQ ID NO: 1 - protein, 166 aa, Homo sapiens
CNLSQTHSLNNRRTLMLMAQMRRISPFSCLKDRHDFEFPQEEFDGNQFQKAQAISVLHEMMQQTFNLFSTKNSSAAWDETLLEKFYIELFQQMNDLEACVIQEVGVEETPLMNEDSILAVKKYFQRITLYLMEKKYSPCAWEVVRAEIMRSLSFSTNLQKRLRRKD

SEQ ID NO: 2 - protein, 166 aa, Homo sapiens
CDLPQTHSLGNRRALILLGQMGRISPFSCLKDRHDFRIPQEEFDGNQFQKAQAISVLHEMMQQTFNLFSTENSSAAWEQTLLEKFSIELFQQMNDLEACVIQEVGVEETPLMNEDSILAVRKYFQRITLYLIERKYSPCAWEVVRAEIMRSLSFSTNLQKRLRRKD

SEQ ID NO: 3 - protein, 166 aa, Homo sapiens
CDLPQTHSLGNRRALILLGQMGRISPFSCLKDRHDFRIPQEEFDGNQFQKAQAISVLHEMMQQTFNLFSTKNSSAAWDETLLEKFYIELFQQMNDLEACVIQEVGVEETPLMNEDSILAVKKYFQRITLYLIERKYSPCAWEVVRAEIMRSLSFSTNLQKRLRRKD